European Patent Application EP 4 349 413 A2, published April 10, 2024. Title: COMBINATION THERAPIES FOR TREATING MYELODYSPLASTIC SYNDROMES AND ACUTE MYELOID LEUKEMIA. Applicant: FORTY SEVEN, INC. The sequence listing filed with the application follows.

SEQUENCE LISTING (153 sequences)

SEQ ID NO: 1 - protein, 5 aa, synthetic construct
  REGION 1..5: note = source = /note="Description of Artificial Sequence: Synthetic peptide"
SYWIT

SEQ ID NO: 2 - protein, 17 aa, synthetic construct
  REGION 1..17: note = source = /note="Description of Artificial Sequence: Synthetic peptide"
DIYPGSGSTNHIEKFKS

SEQ ID NO: 3 - protein, 11 aa, synthetic construct
  REGION 1..11: note = source = /note="Description of Artificial Sequence: Synthetic peptide"
GYGSSYGYFDY

SEQ ID NO: 4 - protein, 11 aa, synthetic construct
  REGION 1..11: note = source = /note="Description of Artificial Sequence: Synthetic peptide"
RASENIYSYLA

SEQ ID NO: 5 - protein, 7 aa, synthetic construct
  REGION 1..7: note = source = /note="Description of Artificial Sequence: Synthetic peptide"
TAKTLAE

SEQ ID NO: 6 - protein, 9 aa, synthetic construct
  REGION 1..9: note = source = /note="Description of Artificial Sequence: Synthetic peptide"
QHQYGPPFT

SEQ ID NO: 7 - protein, 120 aa, synthetic construct
  REGION 1..120: note = source = /note="Description of Artificial Sequence: Synthetic polypeptide"
QVQLVQSGAEVKKPGASVKVSCKASGYTFTSYWITWVKQAPGQGLEWIGDIYPGSGSTNHIEKFKSKATLTVDTSISTAYMELSRLRSDDTAVYYCATGYGSSYGYFDYWGQGTLVTVSS

SEQ ID NO: 8 - protein, 107 aa, synthetic construct
  REGION 1..107: note = source = /note="Description of Artificial Sequence: Synthetic polypeptide"
DIQMTQSPSSLSASVGDRVTITCRASENIYSYLAWYQQKPGKAPKLLIYTAKTLAEGVPSRFSGSGSGTDFTLTISSLQPEDFATYYCQHQYGPPFTFGQGTKLEIK

SEQ ID NO: 9 - protein, 5 aa, synthetic construct
  REGION 1..5: note = source = /note="Description of Artificial Sequence: Synthetic peptide"
SYWMH

SEQ ID NO: 10 - protein, 17 aa, synthetic construct
  REGION 1..17: note = source = /note="Description of Artificial Sequence: Synthetic peptide"
NIDPSDSDTHYNQKFKD

SEQ ID NO: 11 - protein, 10 aa, synthetic construct
  REGION 1..10: note = source = /note="Description of Artificial Sequence: Synthetic peptide"
GYSKYYAMDY

SEQ ID NO: 12 - protein, 16 aa, synthetic construct
  REGION 1..16: note = source = /note="Description of Artificial Sequence: Synthetic peptide"
RSSQSIVHSYGNTYLE

SEQ ID NO: 13 - protein, 7 aa, synthetic construct
  REGION 1..7: note = source = /note="Description of Artificial Sequence: Synthetic peptide"
KVSNRFS

SEQ ID NO: 14 - protein, 9 aa, synthetic construct
  REGION 1..9: note = source = /note="Description of Artificial Sequence: Synthetic peptide"
FQGSHVPYT

SEQ ID NO: 15 - protein, 119 aa, synthetic construct
  REGION 1..119: note = source = /note="Description of Artificial Sequence: Synthetic polypeptide"
QVQLVQSGAEVKKPGASVKVSCKASGYTFTSYWMHWVRQAPGQGLEWMGNIDPSDSDTHYNQKFKDRVTMTRDTSTSTVYMELSSLRSEDTAVYYCARGYSKYYAMDYWGQGTLVTVSS

SEQ ID NO: 16 - protein, 112 aa, synthetic construct
  REGION 1..112: note = source = /note="Description of Artificial Sequence: Synthetic polypeptide"
DIVMTQTPLSLSVTPGQPASISCRSSQSIVHSYGNTYLEWYLQKPGQSPQLLIYKVSNRFSGVPDRFSGSGSGTDFTLKISRVEAEDVGVYYCFQGSHVPYTFGQGTKLEIK

SEQ ID NO: 17 - protein, 449 aa, synthetic construct
  REGION 1..449: note = source = /note="Description of Artificial Sequence: Synthetic polypeptide"
QVQLVQSGAEVKKPGASVKVSCKASGYTFTSYWITWVKQAPGQGLEWIGDIYPGSGSTNHIEKFKSKATLTVDTSISTAYMELSRLRSDDTAVYYCATGYGSSYGYFDYWGQGTLVTVSSASTKGPSVFPLAPSSKSTSGGTAALGCLVKDYFPEPVTVSWNSGALTSGVHTFPAVLQSSGLYSLSSVVTVPSSSLGTQTYICNVNHKPSNTKVDKKVEPKSCDKTHTCPPCPAPELLGGPSVFLFPPKPKDTLMISRTPEVTCVVVDVSHEDPEVKFNWYVDGVEVHNAKTKPREEQYASTYRVVSVLTVLHQDWLNGKEYKCKVSNKALPAPIEKTISKAKGQPREPQVYTLPPSREEMTKNQVSLTCLVKGFYPSDIAVEWESNGQPENNYKTTPPVLDSDGSFFLYSKLTVDKSRWQQGNVFSCSVMHEALHNHYTQKSLSLSPG

SEQ ID NO: 18 - protein, 214 aa, synthetic construct
  REGION 1..214: note = source = /note="Description of Artificial Sequence: Synthetic polypeptide"
DIQMTQSPSSLSASVGDRVTITCRASENIYSYLAWYQQKPGKAPKLLIYTAKTLAEGVPSRFSGSGSGTDFTLTISSLQPEDFATYYCQHQYGPPFTFGQGTKLEIKRTVAAPSVFIFPPSDEQLKSGTASVVCLLNNFYPREAKVQWKVDNALQSGNSQESVTEQDSKDSTYSLSSTLTLSKADYEKHKVYACEVTHQGLSSPVTKSFNRGEC

SEQ ID NO: 19 - protein, 448 aa, synthetic construct
  REGION 1..448: note = source = /note="Description of Artificial Sequence: Synthetic polypeptide"
QVQLVQSGAEVKKPGASVKVSCKASGYTFTSYWMHWVRQAPGQGLEWMGNIDPSDSDTHYNQKFKDRVTMTRDTSTSTVYMELSSLRSEDTAVYYCARGYSKYYAMDYWGQGTLVTVSSASTKGPSVFPLAPSSKSTSGGTAALGCLVKDYFPEPVTVSWNSGALTSGVHTFPAVLQSSGLYSLSSVVTVPSSSLGTQTYICNVNHKPSNTKVDKKVEPKSCDKTHTCPPCPAPELLGGPSVFLFPPKPKDTLMISRTPEVTCVVVDVSHEDPEVKFNWYVDGVEVHNAKTKPREEQYASTYRVVSVLTVLHQDWLNGKEYKCKVSNKALPAPIEKTISKAKGQPREPQVYTLPPSREEMTKNQVSLTCLVKGFYPSDIAVEWESNGQPENNYKTTPPVLDSDGSFFLYSKLTVDKSRWQQGNVFSCSVMHEALHNHYTQKSLSLSPG

SEQ ID NO: 20 - protein, 219 aa, synthetic construct
  REGION 1..219: note = source = /note="Description of Artificial Sequence: Synthetic polypeptide"
DIVMTQTPLSLSVTPGQPASISCRSSQSIVHSYGNTYLEWYLQKPGQSPQLLIYKVSNRFSGVPDRFSGSGSGTDFTLKISRVEAEDVGVYYCFQGSHVPYTFGQGTKLEIKRTVAAPSVFIFPPSDEQLKSGTASVVCLLNNFYPREAKVQWKVDNALQSGNSQESVTEQDSKDSTYSLSSTLTLSKADYEKHKVYACEVTHQGLSSPVTKSFNRGEC

SEQ ID NO: 21 - protein, 5 aa, synthetic construct
  REGION 1..5: note = source = /note="Description of Artificial Sequence: Synthetic peptide"
DYYIH

SEQ ID NO: 22 - protein, 17 aa, synthetic construct
  REGION 1..17: note = source = /note="Description of Artificial Sequence: Synthetic peptide"
RIDPEDGETKYAPKFQG

SEQ ID NO: 23 - protein, 5 aa, synthetic construct
  REGION 1..5: note = source = /note="Description of Artificial Sequence: Synthetic peptide"
GGFAY

SEQ ID NO: 24 - protein, 11 aa, synthetic construct
  REGION 1..11: note = source = /note="Description of Artificial Sequence: Synthetic peptide"
ASSSVSSSYLY

SEQ ID NO: 25 - protein, 7 aa, synthetic construct
  REGION 1..7: note = source = /note="Description of Artificial Sequence: Synthetic peptide"
STSNLAS

SEQ ID NO: 26 - protein, 9 aa, synthetic construct
  REGION 1..9: note = source = /note="Description of Artificial Sequence: Synthetic peptide"
HQWSSHPYT

SEQ ID NO: 27 - protein, 114 aa, synthetic construct
  REGION 1..114: note = source = /note="Description of Artificial Sequence: Synthetic polypeptide"
EVQLQQSGAELVKPGASVKLSCTASGFNIKDYYIHWVKQRTEQGLEWIGRIDPEDGETKYAPKFQGKATITADTSSNTAYLQLNSLTSEDTAVYSCAKGGFAYWGQGTLVTVSA

SEQ ID NO: 28 - protein, 108 aa, synthetic construct
  REGION 1..108: note = source = /note="Description of Artificial Sequence: Synthetic polypeptide"
QIVLTQSPAIMSASPGEKVTLTCSASSSVSSSYLYWYQQKPGSSPKLWIYSTSNLASGVPARFSGSGSGTSYSLTISSMEAEDAASYFCHQWSSHPYTFGGGTKLEIK

SEQ ID NO: 29 - protein, 5 aa, synthetic construct
  REGION 1..5: note = source = /note="Description of Artificial Sequence: Synthetic peptide"
SYWMH

SEQ ID NO: 30 - protein, 17 aa, synthetic construct
  REGION 1..17: note = source = /note="Description of Artificial Sequence: Synthetic peptide"
NIDPSDSDTHYNQKFKD

SEQ ID NO: 31 - protein, 12 aa, synthetic construct
  REGION 1..12: note = source = /note="Description of Artificial Sequence: Synthetic peptide"
SYGNYGENAMDY

SEQ ID NO: 32 - protein, 16 aa, synthetic construct
  REGION 1..16: note = source = /note="Description of Artificial Sequence: Synthetic peptide"
RSSQSIVHSYGNTYLE

SEQ ID NO: 33 - protein, 7 aa, synthetic construct
  REGION 1..7: note = source = /note="Description of Artificial Sequence: Synthetic peptide"
KVSNRFS

SEQ ID NO: 34 - protein, 9 aa, synthetic construct
  REGION 1..9: note = source = /note="Description of Artificial Sequence: Synthetic peptide"
FQGSHVPFT

SEQ ID NO: 35 - protein, 120 aa, synthetic construct
  REGION 1..120: note = source = /note="Description of Artificial Sequence: Synthetic polypeptide"
QVKLQESGAELVRPGSSVKLSCKASGYTFTSYWMHWVKQRPIQGLEWIGNIDPSDSDTHYNQKFKDKATLTVDNSSSTAYMQLSSLTSEDSAVYYCASYGNYGENAMDYWGQGTSVTVSS

SEQ ID NO: 36 - protein, 112 aa, synthetic construct
  REGION 1..112: note = source = /note="Description of Artificial Sequence: Synthetic polypeptide"
DILMTQTPLSLPVSLGDQASISCRSSQSIVHSYGNTYLEWYLQKPGQSPKLLIYKVSNRFSGVPDRFSGSGSGTDFTLKISRVEAEDLGVYYCFQGSHVPFTFGSGTKLEIK

SEQ ID NO: 37 - DNA, 1347 bp, synthetic construct
  misc_feature 1..1347: note = source = /note="Description of Artificial Sequence: Synthetic polynucleotide"
  source 1..1347: mol_type = other DNA
caggttcagttggttcagtctggcgccgaagtgaagaaacctggcgcctctgtgaaggtgtcctgcaaggcttccggctacacctttaccagctactggatcacctgggtcaagcaggctcctggacagggactcgagtggatcggcgatatctatcctggctccggctccaccaaccacatcgagaagttcaagtccaaggctaccctgaccgtggacacctccatctccaccgcctacatggaactgtcccggctgagatctgacgacaccgccgtgtactattgcgctaccggctacggctcctcctacggctactttgattattggggccagggcaccctggtcaccgtgtcctctgcttctaccaagggacccagcgtgttccctctggctccttccagcaagtctacctctggcggaacagctgctctgggctgcctggtcaaggactactttcctgagcctgtgaccgtgtcttggaactctggcgctctgacatctggcgtgcacacattccctgctgtgctgcagtcctccggcctgtactctctgtcctctgtcgtgaccgtgccttccagctctctgggaacccagacctacatctgcaatgtgaaccacaagccttccaacaccaaggtggacaagaaggtggaacccaagtcctgcgacaagacccacacctgtcctccatgtcctgctccagaactgctcggcggaccttccgtgtttctgttccctccaaagcctaaggacaccctgatgatctctcggacccctgaagtgacctgcgtggtggtggatgtgtctcacgaggacccagaagtgaagttcaattggtacgtggacggcgtggaagtgcacaacgccaagaccaagcctagagaggaacagtacgcctccacctacagagtggtgtccgtgctgacagtgctgcaccaggattggctgaacggcaaagagtacaagtgcaaggtgtccaacaaggccctgcctgctcctatcgaaaagaccatctccaaggccaagggccagcctagggaaccccaggtttacaccctgccacctagccgggaagagatgaccaagaaccaggtgtccctgacctgcctcgtgaagggcttctacccttccgatatcgctgtggaatgggagagcaacggccagcctgagaacaactacaagacaacccctcctgtgctggactccgacggctcattctttctgtactccaagctgactgtggacaagtccagatggcagcagggcaacgtgttctcctgcagcgtgatgcacgaggccctgcacaatcactacacacagaagtctctgtctctgagccccggc

SEQ ID NO: 38 - DNA, 642 bp, synthetic construct
  misc_feature 1..642: note = source = /note="Description of Artificial Sequence: Synthetic polynucleotide"
  source 1..642: mol_type = other DNA
gacatccagatgacccagtctccatcctctctgtccgcctctgtgggcgacagagtgaccatcacctgtcgggcctccgagaacatctactcctacctggcctggtatcagcagaagcctggcaaggctcccaagctgctgatctacaccgctaagacactggccgagggcgtgccctctagattttctggctctggaagcggcaccgactttaccctgacaatctccagcctgcagcctgaggacttcgccacctactactgccagcaccagtacggccctccattcacctttggccagggcaccaagctggaaatcaagcggacagtggccgctccttccgtgttcatcttcccaccttccgacgagcagctgaagtctggcacagcctctgtcgtgtgcctgctgaacaacttctaccctcgggaagccaaggtgcagtggaaggtggacaatgccctgcagtccggcaactcccaagagtctgtgaccgagcaggactccaaggacagcacctacagcctgtcctccacactgaccctgtccaaggccgactacgagaagcacaaggtgtacgcctgcgaagtgacccatcagggcctgtctagccctgtgaccaagtctttcaaccggggcgagtgc

SEQ ID NO: 39 - DNA, 1344 bp, synthetic construct
  misc_feature 1..1344: note = source = /note="Description of Artificial Sequence: Synthetic polynucleotide"
  source 1..1344: mol_type = other DNA
caggttcagttggttcagtctggcgccgaagtgaagaaacctggcgcctctgtgaaggtgtcctgcaaggcttccggctacacctttaccagctactggatgcactgggtccgacaggctccaggacaaggcttggagtggatgggcaacatcgacccctctgacagcgacacccactacaaccagaaattcaaggaccgcgtgaccatgaccagagacacctccaccagcaccgtgtacatggaactgtccagcctgagatccgaggacaccgccgtgtactactgtgccagaggctactccaagtactacgccatggactactggggccagggcacactggttaccgtgtcctctgcttccaccaagggaccctctgtgttccctctggctccttccagcaagtctacctctggcggaacagctgctctgggctgcctggtcaaggactactttcctgagcctgtgaccgtgtcttggaactctggcgctctgacatctggcgtgcacacattccctgctgtgctgcagtcctccggcctgtactctctgtcctctgtcgtgaccgtgccttccagctctctgggaacccagacctacatctgcaatgtgaaccacaagccttccaacaccaaggtggacaagaaggtggaacccaagtcctgcgacaagacccacacctgtcctccatgtcctgctccagaactgctcggcggaccttccgtgtttctgttccctccaaagcctaaggacaccctgatgatctctcggacccctgaagtgacctgcgtggtggtggatgtgtcccacgaagatccagaagtgaagttcaattggtacgtggacggcgtggaagtgcacaacgccaagaccaagcctagagaggaacagtacgcctccacctacagagtggtgtccgtgctgacagtgctgcaccaggattggctgaacggcaaagagtacaagtgcaaggtgtccaacaaggccctgcctgctcctatcgaaaagaccatctccaaggccaagggccagcctagggaaccccaggtttacaccctgcctccaagccgggaagagatgaccaagaaccaggtgtccctgacctgcctcgtgaagggcttctacccttccgatatcgccgtggaatgggagagcaatggccagccagagaacaactacaagacaacccctcctgtgctggactccgacggctcattctttctgtactccaagctgaccgtggacaagtccagatggcagcagggcaacgtgttctcctgcagcgtgatgcacgaggccctgcacaatcactatacccagaagtccctgtctctgtcccctggc

SEQ ID NO: 40 - DNA, 657 bp, synthetic construct
  misc_feature 1..657: note = source = /note="Description of Artificial Sequence: Synthetic polynucleotide"
  source 1..657: mol_type = other DNA
gacatcgtgatgacccagacacctctgagcctgagcgtgacacctggacagcctgcctccatctcctgcagatcctctcagtccatcgtgcactcctacggcaacacctacctggaatggtatctgcagaagcccggccagtctcctcagctgctgatctacaaggtgtccaaccggttctctggcgtgcccgacagattttccggctctggctctggcaccgacttcaccctgaagatctccagagtggaagccgaggacgtgggcgtgtactactgcttccaaggctctcacgtgccctacacctttggccagggcaccaagctggaaatcaagcggacagtggccgctccttccgtgttcatcttcccaccttccgacgagcagctgaagtccggcacagcttctgtcgtgtgcctgctgaacaacttctaccctcgggaagccaaggtgcagtggaaggtggacaatgccctgcagtccggcaactcccaagagtctgtgaccgagcaggactccaaggacagcacctacagcctgtccagcacactgaccctgtccaaggccgactacgagaagcacaaggtgtacgcctgcgaagtgacccatcagggcctgtctagccctgtgaccaagtctttcaaccggggcgagtgc

SEQ ID NO: 41 - DNA, 342 bp, synthetic construct
  misc_feature 1..342: note = source = /note="Description of Artificial Sequence: Synthetic polynucleotide"
  source 1..342: mol_type = other DNA
gaggttcagctgcagcagtctggggcagagcttgtgaagccaggggcctcagtcaagttgtcctgcacagcttctggcttcaacattaaagactactatatacactgggtgaagcagaggactgaacagggcctggagtggattggaaggattgatcctgaggatggtgaaactaaatatgccccgaaattccagggcaaggccactataacagcagacacatcctccaacacagcctacctgcagctcaacagcctgacatctgaggacactgccgtctattcctgtgctaagggggggtttgcttactggggccaagggactctggtcactgtctctgca

SEQ ID NO: 42 - DNA, 324 bp, synthetic construct
  misc_feature 1..324: note = source = /note="Description of Artificial Sequence: Synthetic polynucleotide"
  source 1..324: mol_type = other DNA
caaattgttctcacccagtctccagcaatcatgtctgcatctcctggggagaaggtcaccttgacctgcagtgccagttcaagtgtaagttccagctacttgtactggtaccagcagaagccaggatcctcccccaaactctggatttatagcacatccaacctggcttctggagtccctgctcgcttcagtggcagtgggtctgggacctcttactctctcacaatcagcagcatggaggctgaagatgctgcctcttatttctgccatcagtggagtagtcacccgtacacgttcggaggggggaccaagctggaaataaaa

SEQ ID NO: 43 - DNA, 360 bp, synthetic construct
  misc_feature 1..360: note = source = /note="Description of Artificial Sequence: Synthetic polynucleotide"
  source 1..360: mol_type = other DNA
caggtcaagctgcaggagtctggggctgagctggtgaggcctgggtcttcagtgaagctgtcctgcaaggcttctggctacaccttcaccagctactggatgcattgggtgaagcagaggcctatacaaggccttgaatggattggtaacattgacccttctgatagtgatactcactacaatcaaaagttcaaggacaaggccacattgactgtggacaactcctccagcacagcctacatgcagctcagcagcctgacctctgaggactctgcggtctattactgtgcaagctatggtaactacggggagaatgctatggactactggggtcaaggaacctcagtcaccgtctcctca

SEQ ID NO: 44 - DNA, 336 bp, synthetic construct
  misc_feature 1..336: note = source = /note="Description of Artificial Sequence: Synthetic polynucleotide"
  source 1..336: mol_type = other DNA
gatattttgatgacccaaactccactctccctgcctgtcagtcttggagatcaagcctccatctcttgcagatctagtcagagcattgtacatagttatggaaacacctatttagaatggtacctgcagaaaccaggccagtctccaaaactcctgatctacaaagtttccaaccgattttctggggtcccagacaggttcagtggcagtggatcaggtacagatttcacactcaagatcagcagagtggaggctgaggatctgggagtttattactgctttcaaggttcacatgttccattcacgttcggctcggggacaaagttggaaataaaa

SEQ ID NO: 45 - protein, 116 aa, Homo sapiens
EEELQVIQPDKSVLVAAGETATLRCTATSLIPVGPIQWFRGAGPGRELIYNQKEGHFPRVTTVSDLTKRNNMDFSIRIGNITPADAGTYYCVKFRKGSPDDVEFKSGAGTELSVRA

SEQ ID NO: 46 - protein, 113 aa, synthetic construct
  REGION 1..113: note = source = /note="Description of Artificial Sequence: Synthetic polypeptide"
EVQLVQSGAEVKKPGATVKISCKVSGFNIKDYYIHWVQQAPGKGLEWIGRIDPEDGETKYAPKFQDRATITADTSTDTAYMELSSLRSEDTAVYYCARWGAYWGQGTLVTVSS

SEQ ID NO: 47 - protein, 108 aa, synthetic construct
  REGION 1..108: note = source = /note="Description of Artificial Sequence: Synthetic polypeptide"
QIVLTQSPPTLSLSPGERVTLTCSASSSVSSSYLYWYQQKPGQAPKLWIYSTSNLASGVPARFSGSGSGTSYTLTISSLQPEDFAVYFCHQWSSYPRTFGAGTKLEIK

SEQ ID NO: 48 - protein, 116 aa, Homo sapiens; identical to SEQ ID NO: 45

SEQ ID NO: 49 - protein, 115 aa, Homo sapiens
EEELQVIQPDKSVSVAAGESAILHCTVTSLIPVGPIQWFRGAGPARELIYNQKEGHFPRVTTVSESTKRENMDFSISISNITPADAGTYYCVKFRKGSPDTEFKSGAGTELSVRA

SEQ ID NO: 50 - protein, 444 aa, synthetic construct
  REGION 1..444: note = source = /note="Description of Artificial Sequence: Synthetic polypeptide"
QVQLVQSGAEVKKPGASVKVSCKASGYTFTNYNMHWVRQAPGQRLEWMGTIYPGNDDTSYNQKFKDRVTITADTSASTAYMELSSLRSEDTAVYYCARGGYRAMDYWGQGTLVTVSSASTKGPSVFPLAPCSRSTSESTAALGCLVKDYFPEPVTVSWNSGALTSGVHTFPAVLQSSGLYSLSSVVTVPSSSLGTKTYTCNVDHKPSNTKVDKRVESKYGPPCPPCPAPEFLGGPSVFLFPPKPKDTLMISRTPEVTCVVVDVSQEDPEVQFNWYVDGVEVHNAKTKPREEQFNSTYRVVSVLTVLHQDWLNGKEYKCKVSNKGLPSSIEKTISKAKGQPREPQVYTLPPSQEEMTKNQVSLTCLVKGFYPSDIAVEWESNGQPENNYKTTPPVLDSDGSFFLYSRLTVDKSRWQEGNVFSCSVMHEALHNHYTQKSLSLSLGK

SEQ ID NO: 51 - protein, 219 aa, synthetic construct
  REGION 1..219: note = source = /note="Description of Artificial Sequence: Synthetic polypeptide"
DIVMTQSPLSLPVTPGEPASISCRSSQSIVYSNGNTYLGWYLQKPGQSPQLLIYKVSNRFSGVPDRFSGSGSGTDFTLKISRVEAEDVGVYYCFQGSHVPYTFGQGTKLEIKRTVAAPSVFIFPPSDEQLKSGTASVVCLLNNFYPREAKVQWKVDNALQSGNSQESVTEQDSKDSTYSLSSTLTLSKADYEKHKVYACEVTHQGLSSPVTKSFNRGEC

SEQ ID NO: 52 - protein, 5 aa, synthetic construct
  REGION 1..5: note = source = /note="Description of Artificial Sequence: Synthetic peptide"
NYNMH

SEQ ID NO: 53 - protein, 17 aa, synthetic construct
  REGION 1..17: note = source = /note="Description of Artificial Sequence: Synthetic peptide"
TIYPGNDDTSYNQKFKD

SEQ ID NO: 54 - protein, 8 aa, synthetic construct
  REGION 1..8: note = source = /note="Description of Artificial Sequence: Synthetic peptide"
GGYRAMDY

SEQ ID NO: 55 - protein, 15 aa, synthetic construct
  REGION 1..15: note = source = /note="Description of Artificial Sequence: Synthetic peptide"
RSSQSIVYSNGNTYL

SEQ ID NO: 56 - protein, 7 aa, synthetic construct
  REGION 1..7: note = source = /note="Description of Artificial Sequence: Synthetic peptide"
KVSNRFS

SEQ ID NO: 57 - protein, 9 aa, synthetic construct
  REGION 1..9: note = source = /note="Description of Artificial Sequence: Synthetic peptide"
FQGSHVPYT

SEQ ID NO: 58 - protein, 116 aa, synthetic construct
  REGION 1..116: note = source = /note="Description of Artificial Sequence: Synthetic polypeptide"
QVQLQQPGAELVKPGASVMMSCKASGYTFTNYNMHWVKQTPGQGLEWIGTIYPGNDDTSYNQKFKDKATLTADKSSSAAYMQLSSLTSEDSAVYYCARGGYRAMDYWGQTSVTVSS

SEQ ID NO: 59 - protein, 112 aa, synthetic construct
  REGION 1..112: note = source = /note="Description of Artificial Sequence: Synthetic polypeptide"
DVLMTQTPLSLPVSLGDQASISCRSSQSIVYSNGNTYLGWYLQKPGQSPKLLIYKVSNRFSGVPDRFSGSGSGTDFTLKISRVEAEDLGVYHCFQGSHVPYTFGGGTKVEIK

SEQ ID NO: 60 - protein, 118 aa, synthetic construct
  REGION 1..118: note = source = /note="Description of Artificial Sequence: Synthetic polypeptide"
EVQLVESGGGLVQPGGSLRLSCAASGFTFSGYGMSWVRQAPGKGLEWVATITSGGTYTYYPDSVKGRFTISRDNAKNSLYLQMNSLRAEDTAVYYCARSLAGNAMDYWGQGTLVTVSS

SEQ ID NO: 61 - protein, 107 aa, synthetic construct
  REGION 1..107: note = source = /note="Description of Artificial Sequence: Synthetic polypeptide"
EIVLTQSPATLSLSPGERATLSCRASQTISDYLHWYQQKPGQAPRLLIKFASQSISGIPARFSGSGSGTDFTLTISSLEPEDFAVYYCQNGHGFPRTFGQGTKVEIK

SEQ ID NO: 62 - protein, 109 aa, synthetic construct
  REGION 1..109: note = source = /note="Description of Artificial Sequence: Synthetic polypeptide"
EVQLVESGGGLVQPGGSLRLSCAASGFTFSSYWMSWVRQAPGKGLEWVANIKQDGSEKYYVDSVKGRFTISRDNAKNSLYLQMNSLRAEDTAVYYCARWGQGTLVTVSS

SEQ ID NO: 63 - protein, 107 aa, synthetic construct
  REGION 1..107: note = source = /note="Description of Artificial Sequence: Synthetic polypeptide"
DIVMTQSPATLSVTPGDRVSLSCRASQNFSDYLHWYQQKSHESPRLLIKYVSHSISGIPSRFSGSGSGSDFTLSINSVEPEDVGVYYCQNGHSFPPTFGGGTKLEIK

SEQ ID NO: 64 - protein, 116 aa, synthetic construct
  REGION 1..116: note = source = /note="Description of Artificial Sequence: Synthetic polypeptide"
QVQLQQSGAELVKPGASVKLSCKASGYTFTNYYIFWVKERPGQGLEWIGDINPSNGDTNFNEKFKIKATLTVDKSSSTTYMQLNSLTSEDSAVYFCTRGGYTMDYWGQGTSVTVSS

SEQ ID NO: 65 - protein, 112 aa, synthetic construct
  REGION 1..112: note = source = /note="Description of Artificial Sequence: Synthetic polypeptide"
DVVMTQTPLSLPVSLGDQASISCRSSQSLVHSNGNTYFHWYVQKPGQSPKLLIYKVSYRFSGVPDRFSGSGSGTDFTLKISRVEAEDLGVYFCSQSTHVPRTFGGGTKLEIK

SEQ ID NO: 66 - protein, 116 aa, synthetic construct
  REGION 1..116: note = source = /note="Description of Artificial Sequence: Synthetic polypeptide"
QVQLVQSGAEVKKPGASVKVSCKASGYTFTNYYIFWVRQAPGQGLEWIGDINPSNGDTNFNEKFKIKATLTVDKSTSTTYMELSSLRSEDTAVYYCTRGGYTMDYWGQGTLVTVSS

SEQ ID NO: 67 - protein, 116 aa, synthetic construct
  REGION 1..116: note = source = /note="Description of Artificial Sequence: Synthetic polypeptide"
QVQLVQSGAEVKKPGASVKVSCKASGYTFTNYYIFWVRQAPGQGLEWMGDINPSNGDTNFNEKFKIRVTMTRDTSTSTVYMELSSLRSEDTAVYYCTRGGYTMDYWGQGTLVTVSS

SEQ ID NO: 68 - protein, 112 aa, synthetic construct
  REGION 1..112: note = source = /note="Description of Artificial Sequence: Synthetic polypeptide"
DVVMTQTPLSLSVTPGQPASISCRSSQSLVHSNGNTYFHWYLQKPGQPPKLLIYKVSYRFSGVPDRFSGSGSGTDFTLKISRVEAEDVGVYFCSQSTHVPRTFGQGTKVEIK

SEQ ID NO: 69 - protein, 112 aa, synthetic construct
  REGION 1..112: note = source = /note="Description of Artificial Sequence: Synthetic polypeptide"
DIVMTQTPLSLSVTPGQPASISCRSSQSLVHSNGNTYFHWYLQKPGQPPQLLIYKVSYRFSGVPDRFSGSGSGTDFTLKISRVEAEDVGVYYCSQSTHVPRTFGQGTKVEIK

SEQ ID NO: 70 - protein, 118 aa, synthetic construct
  REGION 1..118: note = source = /note="Description of Artificial Sequence: Synthetic polypeptide"
EVQLQQSGAELVRSGASVKLSCTASGFNIKDYYLHWVKQRPEQGLEWIGWIDPDNGDTEFAPKFQGKATMTADTSSNTAYLQLSSLTSEDTAVYYCNAAYGSSSYPMDYWGQGTSVTV

SEQ ID NO: 71 - protein, 118 aa, synthetic construct
  REGION 1..118: note = source = /note="Description of Artificial Sequence: Synthetic polypeptide"
EVQLVQSGAEVKKPGATVKISCKVSGFNIKDYYLHWVQQAPGKGLEWMGWIDPDNGDTEYAEKFQGRVTITADTSTDTAYMELSSLRSEDTAVYYCNAAYGSSSYPMDYWGQGTTVTV

SEQ ID NO: 72 - protein, 118 aa, synthetic construct
  REGION 1..118: note = source = /note="Description of Artificial Sequence: Synthetic polypeptide"
QMQLVQSGAEVKKTGSSVKVSCKASGFNIKDYYLHWVRQAPGQALEWMGWIDPDNGDTEYAQKFQDRVTITRDRSMSTAYMELSSLRSEDTAMYYCNAAYGSSSYPMDYWGQGTTVTV

SEQ ID NO: 73 - protein, 118 aa, synthetic construct
  REGION 1..118: note = source = /note="Description of Artificial Sequence: Synthetic polypeptide"
EVQLVQSGAEVKKTGSSVKVSCKASGFNIKDYYLHWVRQAPGQALEWMGWIDPDNGDTEYAQKFQDRVTITRDRSMSTAYMELSSLRSEDTAMYYCNAAYGSSSYPMDYWGQGTTVTV

SEQ ID NO: 74 - protein, 118 aa, synthetic construct
  REGION 1..118: note = source = /note="Description of Artificial Sequence: Synthetic polypeptide"
QMQLVQSGAEVKKTGSSVKVSCKASGFNIKDYYLHWVRQAPGQALEWMGWIDPDNGDTEYAQKFQGRVTMTADTSSNTAYMELSSLRSEDTAMYYCNAAYGSSSYPMDYWGQGTTVTV

SEQ ID NO: 75 - protein, 118 aa, synthetic construct
  REGION 1..118: note = source = /note="Description of Artificial Sequence: Synthetic polypeptide"
QMQLVQSGAEVKKTGSSVKVSCKASGFNIKDYYLHWVRQAPGQALEWMGWIDPDNGDTEYAQKFQGRVTMTEDTSTDTAYMELSSLRSEDTAMYYCNAAYGSSSYPMDYWGQGTTVTV

SEQ ID NO: 76 - protein, 118 aa, synthetic construct
  REGION 1..118: note = source = /note="Description of Artificial Sequence: Synthetic polypeptide"
QMQLVQSGAEVKKTGSSVKVSCKASGFNIKDYYLHWVRQAPGQALEWMGWIDPDQGDTEYAQKFQDRVTITRDRSMSTAYMELSSLRSEDTAMYYCNAAYGSSSYPMDYWGQGTTVTV

SEQ ID NO: 77 - protein, 118 aa, synthetic construct
  REGION 1..118: note = source = /note="Description of Artificial Sequence: Synthetic polypeptide"
QMQLVQSGAEVKKTGSSVKVSCKASGFNIKDYYLHWVRQAPGQALEWMGWIDPDYGDTEYAQKFQDRVTITRDRSMSTAYMELSSLRSEDTAMYYCNAAYGSSSYPMDYWGQGTTVTV

SEQ ID NO: 78 - protein, 118 aa, synthetic construct
  REGION 1..118: note = source = /note="Description of Artificial Sequence: Synthetic polypeptide"
QMQLVQSGAEVKKTGSSVKVSCKASGFNIKDYYLHWVRQAPGQALEWMGWIDPDSGDTEYAQKFQDRVTITRDRSMSTAYMELSSLRSEDTAMYYCNAAYGSSSYPMDYWGQGTTVTV

SEQ ID NO: 79 - protein, 118 aa, synthetic construct
  REGION 1..118: note = source = /note="Description of Artificial Sequence: Synthetic polypeptide"
QMQLVQSGAEVKKTGSSVKVSCKASGFNIKDYYLHWVRQAPGQALEWMGWIDPDNADTEYAQKFQDRVTITRDRSMSTAYMELSSLRSEDTAMYYCNAAYGSSSYPMDYWGQGTTVTV

SEQ ID NO: 80 - protein, 118 aa, synthetic construct
  REGION 1..118: note = source = /note="Description of Artificial Sequence: Synthetic polypeptide"
QMQLVQSGAEVKKTGSSVKVSCKASGFNIKDYYLHWVRQAPGQALEWMGWIDPDNTDTEYAQKFQDRVTITRDRSMSTAYMELSSLRSEDTAMYYCNAAYGSSSYPMDYWGQGTTVTV

SEQ ID NO: 81 - protein, 118 aa, synthetic construct
  REGION 1..118: note = source = /note="Description of Artificial Sequence: Synthetic polypeptide"
QMQLVQSGAEVKKTGSSVKVSCKASGFNIKDYYLHWVRQAPGQALEWMGWIDPDNGDTEYAQKFQDRVTITRDRSMSTAYMELSSLRSEDTAMYYCNAAYGSSPYPMDYWGQGTTVTV

SEQ ID NO: 82 - protein, 118 aa, synthetic construct
  REGION 1..118: note = source = /note="Description of Artificial Sequence: Synthetic polypeptide"
QMQLVQSGAEVKKTGSSVKVSCKASGYTFTYYYLHWVRQAPGQALEWMGWIDPDNGDTEYAQKFQDRVTITRDRSMSTAYMELSSLRSEDTAMYYCNAAYGSSSYPMDYWGQGTTVTV

SEQ ID NO: 83 - protein, 118 aa, synthetic construct
  REGION 1..118: note = source = /note="Description of Artificial Sequence: Synthetic polypeptide"
QMQLVQSGAEVKKTGSSVKVSCKASGFTFTYYYLHWVRQAPGQALEWMGWIDPDNGDTEYAQKFQDRVTITRDRSMSTAYMELSSLRSEDTAMYYCNAAYGSSSYPMDYWGQGTTVTV

SEQ ID NO: 84 - protein, 118 aa, synthetic construct
  REGION 1..118: note = source = /note="Description of Artificial Sequence: Synthetic polypeptide"
QMQLVQSGAEVKKTGSSVKVSCKASGYNFTYYYLHWVRQAPGQALEWMGWIDPDNGDTEYAQKFQDRVTITRDRSMSTAYMELSSLRSEDTAMYYCNAAYGSSSYPMDYWGQGTTVTV

SEQ ID NO: 85 - protein, 118 aa, synthetic construct
  REGION 1..118: note = source = /note="Description of Artificial Sequence: Synthetic polypeptide"
QMQLVQSGAEVKKTGSSVKVSCKASGYTITYYYLHWVRQAPGQALEWMGWIDPDNGDTEYAQKFQDRVTITRDRSMSTAYMELSSLRSEDTAMYYCNAAYGSSSYPMDYWGQGTTVTV

SEQ ID NO: 86 - protein, 118 aa, synthetic construct
  REGION 1..118: note = source = /note="Description of Artificial Sequence: Synthetic polypeptide"
QMQLVQSGAEVKKTGSSVKVSCKASGYTFKYYYLHWVRQAPGQALEWMGWIDPDNGDTEYAQKFQDRVTITRDRSMSTAYMELSSLRSEDTAMYYCNAAYGSSSYPMDYWGQGTTVTV

SEQ ID NO: 87 - protein, 118 aa, synthetic construct
  REGION 1..118: note = source = /note="Description of Artificial Sequence: Synthetic polypeptide"
QMQLVQSGAEVKKTGSSVKVSCKASGYTFTDYYLHWVRQAPGQALEWMGWIDPDNGDTEYAQKFQDRVTITRDRSMSTAYMELSSLRSEDTAMYYCNAAYGSSSYPMDYWGQGTTVTV

SEQ ID NO: 88 - protein, 118 aa, synthetic construct
  REGION 1..118: note = source = /note="Description of Artificial Sequence: Synthetic polypeptide"
QMQLVQSGAEVKKTGSSVKVSCKASGFTFTDYYLHWVRQAPGQALEWMGWIDPDNGDTEYAQKFQDRVTITRDRSMSTAYMELSSLRSEDTAMYYCNAAYGSSSYPMDYWGQGTTVTV

SEQ ID NO: 89 - protein, 118 aa, synthetic construct
  REGION 1..118: note = source = /note="Description of Artificial Sequence: Synthetic polypeptide"
QMQLVQSGAEVKKTGSSVKVSCKASGFTITDYYLHWVRQAPGQALEWMGWIDPDNGDTEYAQKFQDRVTITRDRSMSTAYMELSSLRSEDTAMYYCNAAYGSSSYPMDYWGQGTTVTV

SEQ ID NO: 90 - protein, 118 aa, synthetic construct
  REGION 1..118: note = source = /note="Description of Artificial Sequence: Synthetic polypeptide"
QMQLVQSGAEVKKTGSSVKVSCKASGYTFKDYYLHWVRQAPGQALEWMGWIDPDNGDTEYAQKFQDRVTITRDRSMSTAYMELSSLRSEDTAMYYCNAAYGSSSYPMDYWGQGTTVTV

SEQ ID NO: 91 - protein, 118 aa, synthetic construct
  REGION 1..118: note = source = /note="Description of Artificial Sequence: Synthetic polypeptide"
QMQLVQSGAEVKKTGSSVKVSCKASGFTFKDYYLHWVRQAPGQALEWMGWIDPDNGDTEYAQKFQDRVTITRDRSMSTAYMELSSLRSEDTAMYYCNAAYGSSSYPMDYWGQGTTVTV

SEQ ID NO: 92 - protein, 118 aa, synthetic construct
  REGION 1..118: note = source = /note="Description of Artificial Sequence: Synthetic polypeptide"
QMQLVQSGAEVKKTGSSVKVSCKASGFNIKDYYLHWVRQAPGQALEWMGWIDPDNGDTEYAQKFQDRVTITRDRSMSTAYLQLSSLRSEDTAMYYCNAAYGSSSYPMDYWGQGTTVTV

SEQ ID NO: 93 - protein, 118 aa, synthetic construct
  REGION 1..118: note = source = /note="Description of Artificial Sequence: Synthetic polypeptide"
QMQLVQSGAEVKKTGSSVKVSCKASGFNIKDYYLHWVRQAPGQALEWMGWIDPDNGDTEYAQKFQDRVTITRDRSMSTAYMELSSLTSEDTAVYYCNAAYGSSSYPMDYWGQGTTVTV

SEQ ID NO: 94 - protein, 118 aa, synthetic construct
  REGION 1..118: note = source = /note="Description of Artificial Sequence: Synthetic polypeptide"
EVQLVQSGAEVKKPGATVKISCKVSGFNIKDYYLHWVRQAPGQALEWMGWIDPDNGDTEYAQKFQDRVTITRDRSMSTAYMELSSLRSEDTAMYYCNAAYGSSSYPMDYWGQGTTVTV

SEQ ID NO: 95 - protein, 118 aa, synthetic construct
  REGION 1..118: note = source = /note="Description of Artificial Sequence: Synthetic polypeptide"
EVQLVQSGAEVKKPGATVKISCKVSGFNIKDYYLHWVQQAPGKGLEWMGWIDPDNGDTEYAQKFQDRVTITRDRSMSTAYMELSSLRSEDTAMYYCNAAYGSSSYPMDYWGQGTTVTV

SEQ ID NO: 96 - protein, 107 aa, synthetic construct
  REGION 1..107: note = source = /note="Description of Artificial Sequence: Synthetic polypeptide"
DIKMTQSPSSLYASLGERVTITCKASQDIHRYLSWFQQKPGKSPKILIYRANRLVDGVPSRFSGSGSGQDYSLTISSLEYEDMGIYYCLQYDEFPYTFGGGTKLEMK

SEQ ID NO: 97 - protein, 107 aa, synthetic construct
  REGION 1..107: note = source = /note="Description of Artificial Sequence: Synthetic polypeptide"
DIKMTQSPSSLYASLGERVTITCKASQDIHRYLSWFQQKPGKSPKILIYRANRLVDGVPSRFSGSGSGQDYSLTISSLEYEDMGIYYCLQYDEFPYTFGGGTKLEIK

SEQ ID NO: 98 - protein, 107 aa, synthetic construct
  REGION 1..107: note = source = /note="Description of Artificial Sequence: Synthetic polypeptide"
DIQMTQSPSSLSASVGDRVTITCKASQDIHRYLSWYQQKPGKAPKLLIYRANRLVDGVPSRFSGSGSGTDFTFTISSLQPEDIATYYCLQYDEFPYTFGGGTKVEIK

SEQ ID NO: 99 - protein, 107 aa, synthetic construct
  REGION 1..107: note = source = /note="Description of Artificial Sequence: Synthetic polypeptide"
DIQMTQSPSSLSASVGDRVTITCKASQDIHRYLSWFQQKPGKAPKSLIYRANRLVDGVPSRFSGSGSGTDFTLTISSLQPEDFATYYCLQYDEFPYTFGGGTKVEIK

SEQ ID NO: 100 - protein, 107 aa, synthetic construct
  REGION 1..107: note = source = /note="Description of Artificial Sequence: Synthetic polypeptide"
NIQMTQSPSAMSASVGDRVTITCKASQDIHRYLSWFQQKPGKVPKHLIYRANRLVDGVPSRFSGSGSGTEFTLTISSLQPEDFATYYCLQYDEFPYTFGGGTKVEIK

SEQ ID NO: 101 - protein, 107 aa, synthetic construct
  REGION 1..107: note = source = /note="Description of Artificial Sequence: Synthetic polypeptide"
DIQMTQSPSSLSASVGDRVTITCKASQDIHRYLSWYQQKPGKAPKRLIYRANRLVDGVPSRFSGSGSGTEFTLTISSLQPEDFATYYCLQYDEFPYTFGGGTKVEIK

SEQ ID NO: 102 - protein, 107 aa, synthetic construct
  REGION 1..107: note = source = /note="Description of Artificial Sequence: Synthetic polypeptide"
DIQMTQSPSSLSASVGDRVTITCRASQDIHRYLAWYQQKPGKVPKLLIYRANRLQSGVPSRFSGSGSGTDFTLTISSLQPEDVATYYCLQYDEFPYTFGQGTKVEIK

SEQ ID NO: 103 - protein, 107 aa, synthetic construct
  REGION 1..107: note = source = /note="Description of Artificial Sequence: Synthetic polypeptide"
EIVLTQSPATLSLSPGERATLSCRASQDIHRYLAWYQQKPGQAPRLLIYRANRRATGIPARFSGSGSGTDFTLTISSLEPEDFAVYYCLQYDEFPYTGFQGTRLEIK

SEQ ID NO: 104 - protein, 107 aa, synthetic construct
  REGION 1..107: note = source = /note="Description of Artificial Sequence: Synthetic polypeptide"
DIQMTQSPSAMSASVGDRVTITCKASQDIHRYLSWFQQKPGKVPKHLIYRANRLVDGVPSRFSGSGSGTEFTLTISSLQPEDFATYYCLQYDEFPYTFGGGTKVEIK

SEQ ID NO: 105 - protein, 107 aa, synthetic construct
  REGION 1..107: note = source = /note="Description of Artificial Sequence: Synthetic polypeptide"
NIQMTQSPSAMSASVGDRVTITCRARQGIHRYLSWFQQKPGKVPKHLIYRANRLVDGVPSRFSGSGSGTEFTLTISSLQPEDFATYYCLQYDEFPYTFGGGTKVEIK

SEQ ID NO: 106 - protein, 107 aa, synthetic construct
  REGION 1..107: note = source = /note="Description of Artificial Sequence: Synthetic polypeptide"
NIQMTQSPSAMSASVGDRVTITCKASQDIHRYLSWFQQKPGKVPKILIYRANRLVDGVPSRFSGSGSGTEFTLTISSLQPEDFATYYCLQYDEFPYTFGGGTKVEIK

SEQ ID NO: 107 - protein, 107 aa, synthetic construct
  REGION 1..107: note = source = /note="Description of Artificial Sequence: Synthetic polypeptide"
NIQMTQSPSAMSASVGDRVTITCKASQDIHRYLSWFQQKPGKVPKHLIYRANRLVSGVPSRFSGSGSGTEFTLTISSLQPEDFATYYCLQYDEFPYTFGGGTKVEIK

SEQ ID NO: 108 - protein, 107 aa, synthetic construct
  REGION 1..107: note = source = /note="Description of Artificial Sequence: Synthetic polypeptide"
NIQMTQSPSAMSASVGDRVTITCRARQGIHRYLSWFQQKPGKVPKILIYRANRLVDGVPSRFSGSGSGTEFTLTISSLQPEDFATYYCLQYDEFPYTFGGGTKVEIK

SEQ ID NO: 109 - protein, 107 aa, synthetic construct
  REGION 1..107: note = source = /note="Description of Artificial Sequence: Synthetic polypeptide"
NIQMTQSPSAMSASVGDRVTITCRARQGIHRYLSWFQQKPGKVPKHLIYRANRLVSGVPSRFSGSGSGTEFTLTISSLQPEDFATYYCLQYDEFPYTFGGGTKVEIK

SEQ ID NO: 110 - protein, 107 aa, synthetic construct
  REGION 1..107: note = source = /note="Description of Artificial Sequence: Synthetic polypeptide"
NIQMTQSPSAMSASVGDRVTITCKASQDIHRYLSWFQQKPGKVPKLLIYRANRLVDGVPSRFSGSGSGTEFTLTISSLQPEDFATYYCLQYDEFPYTFGGGTKVEIK

SEQ ID NO: 111 - protein, 107 aa, synthetic construct
  REGION 1..107: note = source = /note="Description of Artificial Sequence: Synthetic polypeptide"
NIQMTQSPSAMSASVGDRVTITCKASQDIHRYLSWFQQKPGKVPKLLIYRANRLVSGVPSRFSGSGSGTEFTLTISSLQPEDFATYYCLQYDEFPYTFGGGTKVEIK

SEQ ID NO: 112 - protein, 107 aa, synthetic construct
  REGION 1..107: note = source = /note="Description of Artificial Sequence: Synthetic polypeptide"
NIQMTQSPSAMSASVGDRVTITCRARQGIHRYLSWFQQKPGKVPKLLIYRANRLVSGVPSRFSGSGSGTEFTLTISSLQPEDFATYYCLQYDEFPYTFGGGTKVEIK

SEQ ID NO: 113 - protein, 117 aa, synthetic construct
  REGION 1..117: note = source = /note="Description of Artificial Sequence: Synthetic polypeptide"
QVQLVQSGAEVKKPGASVKVSCKASGYTFTNYNMHWVRQAPGQGLEWIGTIYPGNDDTSYNQKFKDKATLTADKSTSTAYMELSSLRSEDTAVYYCARGGYRAMDYWGQGTLVTVSS

SEQ ID NO: 114 - protein, 117 aa, synthetic construct
  REGION 1..117: note = source = /note="Description of Artificial Sequence: Synthetic polypeptide"
QVQLVQSGAEVKKPGASVKVSCKASGYTFTNYNMHWVRQAPGQRLEWMGTIYPGNDDTSYNQKFKDRVTITADTSASTAYMELSSLRSEDTAVYYCARGGYRAMDYWGQGTLVTVSS

SEQ ID NO: 115 - protein, 117 aa, synthetic construct
  REGION 1..117: note = source = /note="Description of Artificial Sequence: Synthetic polypeptide"
QVQLVQSGAEVKKPGASVKVSCKASGYTFTNYNMHWVRQAPGQRLEWIGTIYPGNDDTSYNQKFKDRATLTADKSASTAYMELSSLRSEDTAVYYCARGGYRAMDYWGQGTLVTVSS

SEQ ID NO: 116 - protein, 112 aa, synthetic construct
  REGION 1..112: note = source = /note="Description of Artificial Sequence: Synthetic polypeptide"
DVVMTQSPLSLPVTPGEPASISCRSSQSIVYSNGNTYLGWYLQKPGQSPKLLIYKVSNRFSGVPDRFSGSGSGTDFTLKISRVEAEDVGVYHCFQGSHVPYTFGGGTKVEIK

SEQ ID NO: 117 - protein, 112 aa, synthetic construct
  REGION 1..112: note = source = /note="Description of Artificial Sequence: Synthetic polypeptide"
DIVMTQSPLSLPVTPGEPASISCRSSQSIVYSNGNTYLGWYLQKPGQSPQLLIYKVSNRFSGVPDRFSGSGSGTDFTLKISRVEAEDVGVYYCFQGSHVPYTFGQGTKLEIK

SEQ ID NO: 118 - protein, 112 aa, synthetic construct
  REGION 1..112: note = source = /note="Description of Artificial Sequence: Synthetic polypeptide"
DVVMTQSPLSLPVTPGEPASISCRSSQSIVYSNGNTYLGWYLQKPGQSPQLLIYKVSNRFSGVPDRFSGSGSGTDFTLKISRVEAEDVGVYHCFQGSHVPYTFGQGTKLEIK

SEQ ID NO: 119 - protein, 120 aa, synthetic construct
  REGION 1..120: note = source = /note="Description of Artificial Sequence: Synthetic polypeptide"
QVQLQQPGAELVRPGSSVKLSCKASGYTFTSYWVHWVKQRPIQGLEWIGNIDPSDSDTHYNQKFKDKASLTVDKSSSTAYMQLSSLTFEDSAVYYCVRGGTGTMAWFAYWGQGTLVTVSA

SEQ ID NO: 120 - protein, 120 aa, synthetic construct
  REGION 1..120: note = source = /note="Description of Artificial Sequence: Synthetic polypeptide"
EVQLVQSGAEVKKPGESLRISCKASGYTFTSYWVHWVRQMPGKGLEWIGNIDPSDSDTHYNQKFKDHVTLSVDKSISTAYLQLSSLKASDTAMYYCVRGGTGTMAWFAYWGQGTLVTVSS

SEQ ID NO: 121 - protein, 120 aa, synthetic construct
  REGION 1..120: note = source = /note="Description of Artificial Sequence: Synthetic polypeptide"
EVQLVQSGAEVKKPGESLRISCKASGYSFTSYWVHWVRQMPGKGLEWMGNIDPSDSDTHYNQKFKDHVTLSVDKSISTAYLQLSSLKASDTAMYYCVRGGTGTMAWFAYWGQGTLVTVSS

SEQ ID NO: 122 - protein, 120 aa, synthetic construct
  REGION 1..120: note = source = /note="Description of Artificial Sequence: Synthetic polypeptide"
EVQLVQSGAEVKKPGESLRISCKASGYSFTSYWVHWVRQMPGKGLEWMGNIDPSDSDTHYSPSFQGHVTLSVDKSISTAYLQLSSLKASDTAMYYCVRGGTGTMAWFAYWGQGTLVTVSS

SEQ ID NO: 123 - protein, 120 aa, synthetic construct
  REGION 1..120: note = source = /note="Description of Artificial Sequence: Synthetic polypeptide"
EVQLVQSGAEVKKPGESLRISCKASGYSFTSYWVHWVRQMPGKGLEWMGNIDPSDSDTHYSPSFQGHVTLSVDKSISTAYLQLSSLKASDTAMYYCVRGGTGTLAWFAYWGQGTLVTVSS

SEQ ID NO: 124 - protein, 120 aa, synthetic construct
  REGION 1..120: note = source = /note="Description of Artificial Sequence: Synthetic polypeptide"
EVQLVQSGAEVKKPGESLRISCKASGYSFTSYWVHWVRQMPGKGLEWMGNIDPSDSDTHYSPSFQGHVTLSVDKSISTAYLQLSSLKASDTAMYYCVRGGTGTMAYFAYWGQGTLVTVSS

SEQ ID NO: 125 - protein, 120 aa, synthetic construct
  REGION 1..120: note = source = /note="Description of Artificial Sequence: Synthetic polypeptide"
EVQLVQSGAEVKKPGESLRISCKASGYSFTSYWVHWVRQMPGKGLEWMGNIDPSDSDTHYSPSFQGHVTLSVDKSISTAYLQLSSLKASDTAMYYCVRGGTGTLAYFAYWGQGTLVTVSS

SEQ ID NO: 126 - protein, 112 aa, synthetic construct
  REGION 1..112: note = source = /note="Description of Artificial Sequence: Synthetic polypeptide"
DVVMTQTPLSLPVSLGDQASISCRSSQSLVHSYGNTYLYWYLQKPGQSPKLLIYRVSNRFSGVPDRFSGSGSGTDFTLKISRVEAEDLGVYFCFQGTHVPYTFGSGTKLEIK

SEQ ID NO: 127 - protein, 112 aa, synthetic construct
  REGION 1..112: note = source = /note="Description of Artificial Sequence: Synthetic polypeptide"
DVVMTQSPLSLPVTLGQPASISCRSSQSLVHSYGNTYLYWYQQRPGQSPRLLIYRVSNRFSGVPDRFSGSGSGTDFTLKISRVEAEDVGVYFCFQGTHVPYTFGGGTKVEIK

SEQ ID NO: 128 - protein, 112 aa, synthetic construct
  REGION 1..112: note = source = /note="Description of Artificial Sequence: Synthetic polypeptide"
DVVMTQSPLSLPVTLGQPASISCRSSQSLVHSYGNTYLYWFQQRPGQSPRLLIYRVSNRFSGVPDRFSGSGSGTDFTLKISRVEAEDVGVYYCFQGTHVPYTFGGGTKVEIK

SEQ ID NO: 129 - protein, 393 aa, Homo sapiens [sequence omitted]

SEQ ID NO: 130 - DNA, 2512 bp, Homo sapiens
  source 1..2512: mol_type = unassigned DNA
ctcaaaagtctagagccaccgtccagggagcaggtagctgctgggctccggggacactttgcgttcgggctgggagcgtgctttccacgacggtgacacgcttccctggattggcagccagactgccttccgggtcactgccatggaggagccgcagtcagatcctagcgtcgagccccctctgagtcaggaaacattttcagacctatggaaactacttcctgaaaacaacgttctgtcccccttgccgtcccaagcaatggatgatttgatgctgtccccggacgatattgaacaatggttcactgaagacccaggtccagatgaagctcccagaatgccagaggctgctccccccgtggcccctgcaccagcagctcctacaccggcggcccctgcaccagccccctcctggcccctgtcatcttctgtcccttcccagaaaacctaccagggcagctacggtttccgtctgggcttcttgcattctgggacagccaagtctgtgacttgcacgtactcccctgccctcaacaagatgttttgccaactggccaagacctgccctgtgcagctgtgggttgattccacacccccgcccggcacccgcgtccgcgccatggccatctacaagcagtcacagcacatgacggaggttgtgaggcgctgcccccaccatgagcgctgctcagatagcgatggtctggcccctcctcagcatcttatccgagtggaaggaaatttgcgtgtggagtatttggatgacagaaacacttttcgacatagtgtggtggtgccctatgagccgcctgaggttggctctgactgtaccaccatccactacaactacatgtgtaacagttcctgcatgggcggcatgaaccggaggcccatcctcaccatcatcacactggaagactccagtggtaatctactgggacggaacagctttgaggtgcgtgtttgtgcctgtcctgggagagaccggcgcacagaggaagagaatctccgcaagaaaggggagcctcaccacgagctgcccccagggagcactaagcgagcactgcccaacaacaccagctcctctccccagccaaagaagaaaccactggatggagaatatttcacccttcagatccgtgggcgtgagcgcttcgagatgttccgagagctgaatgaggccttggaactcaaggatgcccaggctgggaaggagccaggggggagcagggctcactccagccacctgaagtccaaaaagggtcagtctacctcccgccataaaaaactcatgttcaagacagaagggcctgactcagactgacattctccacttcttgttccccactgacagcctcccacccccatctctccctcccctgccattttgggttttgggtctttgaacccttgcttgcaataggtgtgcgtcagaagcacccaggacttccatttgctttgtcccggggctccactgaacaagttggcctgcactggtgttttgttgtggggaggaggatggggagtaggacataccagcttagattttaaggtttttactgtgagggatgtttgggagatgtaagaaatgttcttgcagttaagggttagtttacaatcagccacattctaggtaggggcccacttcaccgtactaaccagggaagctgtccctcactgttgaattttctctaacttcaaggcccatatctgtgaaatgctggcatttgcacctacctcacagagtgcattgtgagggttaatgaaataatgtacatctggccttgaaaccaccttttattacatggggtctagaacttgacccccttgagggtgcttgttccctctccctgttggtcggtgggttggtagtttctacagttgggcagctggttaggtagagggagttgtcaagtctctgctggcccagccaaaccctgtctgacaacctcttggtgaaccttagtacctaaaaggaaatctcaccccatcccacaccctggaggatttcatctcttgtatatgatgatctggatccaccaagacttgttttatgctcagggtcaatttcttttttcttttttttttttttttttctttttctttgagactgggtctcgctttgttgcccaggctggagtggagtggcgtgatcttggcttactgcagcctttgcctccccggctcgagcagtcctgcctcagcctccggagtagctgggaccacaggttcatgccaccatggccagccaacttttgcatgttttgtagagatggggtctcacagtgttgcccaggctggtctcaaactcctgggctcaggcgatccacctgtctcagcctcccagagtgctgggattacaattgtgagccaccacgtccagctggaagggtcaacatcttttacattctgcaagcacatctgcattttcaccccacccttcccctccttctccctttttatatcccatttttatatcgatctcttattttacaataaaactttgctgcca

SEQ ID NO: 131 - protein, 117 aa, synthetic construct; identical to SEQ ID NO: 114
  REGION 1..117: note = source = /note="Description of Artificial Sequence: Synthetic polypeptide"

SEQ ID NO: 132 - protein, 112 aa, synthetic construct; identical to SEQ ID NO: 117
  REGION 1..112: note = source = /note="Description of Artificial Sequence: Synthetic polypeptide"

SEQ ID NO: 133 - protein, 16 aa, synthetic construct
  REGION 1..16: note = source = /note="Description of Artificial Sequence: Synthetic peptide"
RSSQSIVYSNGNTYLG

SEQ ID NO: 134 - protein, 8 aa, synthetic construct
  REGION 1..8: note = source = /note="Description of Artificial Sequence: Synthetic peptide"
GYTFTNYN

SEQ ID NO: 135 - protein, 8 aa, synthetic construct
  REGION 1..8: note = source = /note="Description of Artificial Sequence: Synthetic peptide"
IYPGNDDT

SEQ ID NO: 136 - protein, 10 aa, synthetic construct
  REGION 1..10: note = source = /note="Description of Artificial Sequence: Synthetic peptide"
ARGGYRAMDY

SEQ ID NO: 137 - protein, 11 aa, synthetic construct
  REGION 1..11: note = source = /note="Description of Artificial Sequence: Synthetic peptide"
QSIVYSNGNTY

SEQ ID NO: 138 - skipped

SEQ ID NO: 139 - protein, 9 aa, synthetic construct
  REGION 1..9: note = source = /note="Description of Artificial Sequence: Synthetic peptide"
FQGSHVPYT

SEQ ID NO: 140 - protein, 7 aa, synthetic construct
  REGION 1..7: note = source = /note="Description of Artificial Sequence: Synthetic peptide"
GYTFTNY

SEQ ID NO: 141 - protein, 4 aa, synthetic construct
  REGION 1..4: note = source = /note="Description of Artificial Sequence: Synthetic peptide"
PGND

SEQ ID NO: 142 - protein, 6 aa, synthetic construct
  REGION 1..6: note = source = /note="Description of Artificial Sequence: Synthetic peptide"
GYRAMD

SEQ ID NO: 143 - protein, 12 aa, synthetic construct
  REGION 1..12: note = source = /note="Description of Artificial Sequence: Synthetic peptide"
SQSIVYSNGNTY

SEQ ID NO: 144 - skipped

SEQ ID NO: 145 - protein, 6 aa, synthetic construct
  REGION 1..6: note = source = /note="Description of Artificial Sequence: Synthetic peptide"
GSHVPY

SEQ ID NO: 146 - protein, 10 aa, synthetic construct
  REGION 1..10: note = source = /note="Description of Artificial Sequence: Synthetic peptide"
ASGYTFTNYN

SEQ ID NO: 147 - protein, 17 aa, synthetic construct
  REGION 1..17: note = source = /note="Description of Artificial Sequence: Synthetic peptide"
IYPGNDDTSYNQKFKDR

SEQ ID NO: 148 - protein, 7 aa, synthetic construct
  REGION 1..7: note = source = /note="Description of Artificial Sequence: Synthetic peptide"
GGYRAMD

SEQ ID NO: 149 - protein, 13 aa, synthetic construct
  REGION 1..13: note = source = /note="Description of Artificial Sequence: Synthetic peptide"
SSQSIVYSNGNTY

SEQ ID NO: 150 - protein, 12 aa, synthetic construct
  REGION 1..12: note = source = /note="Description of Artificial Sequence: Synthetic peptide"
KVSNRFSGVPDR

SEQ ID NO: 151 - protein, 6 aa, synthetic construct
  REGION 1..6: note = source = /note="Description of Artificial Sequence: Synthetic peptide"
GSHVPY

SEQ ID NO: 152 - protein, 15 aa, synthetic construct
  REGION 1..15: note = source = /note="Description of Artificial Sequence: Synthetic peptide"
RRCPLYISYDPVCRR

SEQ ID NO: 153 - protein, 19 aa, synthetic construct
  REGION 1..19: note = source = /note="Description of Artificial Sequence: Synthetic peptide"
RRRRCPLYISYDPVCRRRR